European Patent Application EP 4 424 831 A1, published September 4, 2024. Title: 改良型β－フルクトフラノシダーゼ. Applicant: 京都府公立大学法人. The sequence listing filed with the application follows.

SEQUENCE LISTING (41 sequences)

SEQ ID NO: 1 - protein, 654 aa, Aspergillus fijiensis
MKLTTTTLALATGAAAAEASYHLDTTAPPPTNLSTLPNNTLFHVWRPRAHILPAEGQIGDPCAHYTDPSTGLFHVGFLHDGDGIAGATTANLATYTDTSDNGSFLIQPGGKNDPVAVFDGAVIPVGVNNTPTLLYTSVSFLPIHWSIPYTRGSETQSLAVARDGGRRFDKLDQGPVIADHPFAVDVTAFRDPFVFRSAKLDVLLSLDEEVARNETAVQQAVDGWTEKNAPWYVAVSGGVHGVGPAQFLYRQNGGNASEFQYWEYLGEWWQEATNSSWGDEGTWAGRWGFNFETGNVLFLTEEGHDPQTGEVFVTLGTEGSGLPIVPQVSSIHDMLWAAGEVGVGSEQEGAKVEFSPSMAGFLDWGFSAYAAAGKVLPASSAVSKTSGVEVDRYVSFVWLTGDQYEQADGFPTAQQGWTGSLLLPRELKVQTVENVVDNELVREEGVSWVVGESDNQTARLRTLGITIARETKAALLANGSVTAEEDRTLQTAAVVPFAQSPSSKFFVLTAQLEFPASARSSPLQSGFEILASELERTAIYYQFSNESLVVDRSQTSAAAPTNPGLDSFTESGKLRLFDVIENGQEQVETLDLTVVVDNAVVEVYANGRFALSTWARSWYDNSTQIRFFHNGEGEVQFRNVSVSEGLYNAWPERN

SEQ ID NO: 2 - DNA, 42 bp, synthetic construct
  source 1..42: mol_type = other DNA
attataggatcctcctaccatttggatacgactgcaccaccg

SEQ ID NO: 3 - DNA, 45 bp, synthetic construct
  source 1..45: mol_type = other DNA
attatactcgagttatcagttgcgctcaggccacgcgttatataa

SEQ ID NO: 4 - DNA, 30 bp, synthetic construct
  source 1..30: mol_type = other DNA
gctgacggcattgccggtgcaactaccgcc

SEQ ID NO: 5 - DNA, 36 bp, synthetic construct
  source 1..36: mol_type = other DNA
gatgacggcattgccggtgcaactaccgccaacctg

SEQ ID NO: 6 - DNA, 36 bp, synthetic construct
  source 1..36: mol_type = other DNA
gaggacggcattgccggtgcaactaccgccaacctg

SEQ ID NO: 7 - DNA, 36 bp, synthetic construct
  source 1..36: mol_type = other DNA
tttgacggcattgccggtgcaactaccgccaacctg

SEQ ID NO: 8 - DNA, 36 bp, synthetic construct
  source 1..36: mol_type = other DNA
catgacggcattgccggtgcaactaccgccaacctg

SEQ ID NO: 9 - DNA, 36 bp, synthetic construct
  source 1..36: mol_type = other DNA
attgacggcattgccggtgcaactaccgccaacctg

SEQ ID NO: 10 - DNA, 36 bp, synthetic construct
  source 1..36: mol_type = other DNA
aaggacggcattgccggtgcaactaccgccaacctg

SEQ ID NO: 11 - DNA, 36 bp, synthetic construct
  source 1..36: mol_type = other DNA
cttgacggcattgccggtgcaactaccgccaacctg

SEQ ID NO: 12 - DNA, 36 bp, synthetic construct
  source 1..36: mol_type = other DNA
atggacggcattgccggtgcaactaccgccaacctg

SEQ ID NO: 13 - DNA, 36 bp, synthetic construct
  source 1..36: mol_type = other DNA
aatgacggcattgccggtgcaactaccgccaacctg

SEQ ID NO: 14 - DNA, 36 bp, synthetic construct
  source 1..36: mol_type = other DNA
cctgacggcattgccggtgcaactaccgccaacctg

SEQ ID NO: 15 - DNA, 36 bp, synthetic construct
  source 1..36: mol_type = other DNA
caggacggcattgccggtgcaactaccgccaacctg

SEQ ID NO: 16 - DNA, 36 bp, synthetic construct
  source 1..36: mol_type = other DNA
cgtgacggcattgccggtgcaactaccgccaacctg

SEQ ID NO: 17 - DNA, 30 bp, synthetic construct
  source 1..30: mol_type = other DNA
tctgacggcattgccggtgcaactaccgcc

SEQ ID NO: 18 - DNA, 36 bp, synthetic construct
  source 1..36: mol_type = other DNA
actgacggcattgccggtgcaactaccgccaacctg

SEQ ID NO: 19 - DNA, 30 bp, synthetic construct
  source 1..30: mol_type = other DNA
gttgacggcattgccggtgcaactaccgcc

SEQ ID NO: 20 - DNA, 30 bp, synthetic construct
  source 1..30: mol_type = other DNA
tgggacggcattgccggtgcaactaccgcc

SEQ ID NO: 21 - DNA, 30 bp, synthetic construct
  source 1..30: mol_type = other DNA
tatgacggcattgccggtgcaactaccgcc

SEQ ID NO: 22 - DNA, 30 bp, synthetic construct
  source 1..30: mol_type = other DNA
atcatgcaggaatccaacgtgaaaaagtcc

SEQ ID NO: 23 - DNA, 36 bp, synthetic construct
  source 1..36: mol_type = other DNA
gcgccaatccattggagtattccctatacgcgcggt

SEQ ID NO: 24 - DNA, 36 bp, synthetic construct
  source 1..36: mol_type = other DNA
gacccaatccattggagtattccctatacgcgcggt

SEQ ID NO: 25 - DNA, 36 bp, synthetic construct
  source 1..36: mol_type = other DNA
gagccaatccattggagtattccctatacgcgcggt

SEQ ID NO: 26 - DNA, 36 bp, synthetic construct
  source 1..36: mol_type = other DNA
ttcccaatccattggagtattccctatacgcgcggt

SEQ ID NO: 27 - DNA, 36 bp, synthetic construct
  source 1..36: mol_type = other DNA
gggccaatccattggagtattccctatacgcgcggt

SEQ ID NO: 28 - DNA, 36 bp, synthetic construct
  source 1..36: mol_type = other DNA
cacccaatccattggagtattccctatacgcgcggt

SEQ ID NO: 29 - DNA, 36 bp, synthetic construct
  source 1..36: mol_type = other DNA
atcccaatccattggagtattccctatacgcgcggt

SEQ ID NO: 30 - DNA, 36 bp, synthetic construct
  source 1..36: mol_type = other DNA
aagccaatccattggagtattccctatacgcgcggt

SEQ ID NO: 31 - DNA, 36 bp, synthetic construct
  source 1..36: mol_type = other DNA
atgccaatccattggagtattccctatacgcgcggt

SEQ ID NO: 32 - DNA, 36 bp, synthetic construct
  source 1..36: mol_type = other DNA
aacccaatccattggagtattccctatacgcgcggt

SEQ ID NO: 33 - DNA, 36 bp, synthetic construct
  source 1..36: mol_type = other DNA
ccgccaatccattggagtattccctatacgcgcggt

SEQ ID NO: 34 - DNA, 36 bp, synthetic construct
  source 1..36: mol_type = other DNA
cagccaatccattggagtattccctatacgcgcggt

SEQ ID NO: 35 - DNA, 36 bp, synthetic construct
  source 1..36: mol_type = other DNA
cggccaatccattggagtattccctatacgcgcggt

SEQ ID NO: 36 - DNA, 36 bp, synthetic construct
  source 1..36: mol_type = other DNA
tcgccaatccattggagtattccctatacgcgcggt

SEQ ID NO: 37 - DNA, 36 bp, synthetic construct
  source 1..36: mol_type = other DNA
acgccaatccattggagtattccctatacgcgcggt

SEQ ID NO: 38 - DNA, 36 bp, synthetic construct
  source 1..36: mol_type = other DNA
gtgccaatccattggagtattccctatacgcgcggt

SEQ ID NO: 39 - DNA, 36 bp, synthetic construct
  source 1..36: mol_type = other DNA
tggccaatccattggagtattccctatacgcgcggt

SEQ ID NO: 40 - DNA, 36 bp, synthetic construct
  source 1..36: mol_type = other DNA
tacccaatccattggagtattccctatacgcgcggt

SEQ ID NO: 41 - DNA, 36 bp, synthetic construct
  source 1..36: mol_type = other DNA
aaatgagacagatgtatacagcaacgtaggggtatt